European Patent Specification EP 3 538 674 B1, published March 13, 2024. Title: COMPOSITIONS AND METHODS FOR DETECTION OF BK VIRUS. Applicant: Roche Diagnostics GmbH F. Hoffmann-La Roche AG Roche Molecular Systems, Inc. The sequence listing filed with the application follows.

SEQUENCE LISTING (11 sequences)

SEQ ID NO: 1 - DNA, 25 bp, Artificial Sequence
  Primer
  modified_base (25)..(25): t-Butyl Benzyl-dA
cctaactcctcaaacatatgctgta

SEQ ID NO: 2 - DNA, 23 bp, Artificial Sequence
  Primer
  modified_base (23)..(23): t-Butyl Benzyl-dA
acagtggaaactttgtgatccca

SEQ ID NO: 3 - DNA, 27 bp, Artificial Sequence
  Probe
  modified_base (17)..(17): 7-deaza-deoxyguanosine
attgctggtgctcctggggctattgct

SEQ ID NO: 4 - DNA, 23 bp, Artificial Sequence
  Primer
  modified_base (23)..(23): t-Butyl Benzyl-dA
ggctatagctgctataggcctaa

SEQ ID NO: 5 - DNA, 28 bp, Artificial Sequence
  Primer
  modified_base (28)..(28): t-Butyl Benzyl-dC
agtaacagtttgaattaaagcagcaaac

SEQ ID NO: 6 - DNA, 23 bp, Artificial Sequence
  Primer
  modified_base (23)..(23): t-Butyl Benzyl-dC
agaggaaaatcagcacaaacctc

SEQ ID NO: 7 - DNA, 18 bp, Artificial Sequence
  Primer
  modifed_base (18)..(18): t-Butyl Benzyl-dC
caccctgacaaagggggc

SEQ ID NO: 8 - DNA, 34 bp, Artificial Sequence
  Probe
tgagctactccaggttccaaaatcaggctgatga

SEQ ID NO: 9 - DNA, 28 bp, Artificial Sequence
  Primer
  modified_base (28)..(28): t-Butyl Benzyl-dA
cctttacatcctgctccatttttttata

SEQ ID NO: 10 - DNA, 24 bp, Artificial Sequence
  Primer
  modified_base (24)..(24): t-Butyl Benzyl-dA
agtgtaaggaatttcaccctgaca

SEQ ID NO: 11 - DNA, 38 bp, Artificial Sequence
  Probe
agtattcattctcttcattttatcctcgtcgccccctt